European Patent Application EP 4 279 591 A1, published November 22, 2023. Title: RNA Molecule, Chimeric NA Molecule, Double-Stranded RNA Molecule, and Double-Stranded Chimeric NA Molecule. Applicant: The University of Tokyo. The sequence listing filed with the application follows.

SEQUENCE LISTING (107 sequences)

SEQ ID NO: 1 - RNA, 21 nt, Artificial Sequence
  siRNA passenger strand
gggagcugauggccuaggaaa

SEQ ID NO: 2 - RNA, 21 nt, Artificial Sequence
  siRNA guide strand (6)...(8) 2'-O-methyl modified
uccuaggccaucagcucccac

SEQ ID NO: 3 - RNA, 21 nt, Artificial Sequence
  siRNA guide strand (6) and (8) 2'-O-methyl modified
uccuaggccaucagcucccac

SEQ ID NO: 4 - DNA, 33 bp, Artificial Sequence
  reporter sense strand
tggtagttggagctggtggcgtaggcaagagtg

SEQ ID NO: 5 - DNA, 33 bp, Artificial Sequence
  reporter antisense strand
cactcttgcctacgccaccagctccaactacca

SEQ ID NO: 6 - DNA, 33 bp, Artificial Sequence
  reporter sense strand
tggtagttggagctgatggcgtaggcaagagtg

SEQ ID NO: 7 - DNA, 33 bp, Artificial Sequence
  reporter antisense strand
cactcttgcctacgccatcagctccaactacca

SEQ ID NO: 8 - DNA, 21 bp, Artificial Sequence
  siRNA passenger strand
guuggagcugauggcguagtt

SEQ ID NO: 9 - DNA, 21 bp, Artificial Sequence
  siRNA guide strand
cuacgccaucagcuccaactt

SEQ ID NO: 10 - RNA, 21 nt, Artificial Sequence
  siRNA passenger strand
uuggagcugauggcguaggca

SEQ ID NO: 11 - RNA, 21 nt, Artificial Sequence
  siRNA guide strand
ccuacgccaucagcuccaacu

SEQ ID NO: 12 - RNA, 21 nt, Artificial Sequence
  siRNA passenger strand
uggagcugauggcguaggcaa

SEQ ID NO: 13 - RNA, 21 nt, Artificial Sequence
  siRNA guide strand
gccuacgccaucagcuccaac

SEQ ID NO: 14 - RNA, 21 nt, Artificial Sequence
  siRNA passenger strand
gggagcugauggcguaggaaa

SEQ ID NO: 15 - RNA, 21 nt, Artificial Sequence
  siRNA guide strand
uccuacgccaucagcucccac

SEQ ID NO: 16 - RNA, 21 nt, Artificial Sequence
  siRNA passenger strand
gggagcugauggcguaggaaa

SEQ ID NO: 17 - RNA, 21 nt, Artificial Sequence
  siRNA guide strand (2)...(5) 2'-O-methyl modified
uccuacgccaucagcucccac

SEQ ID NO: 18 - RNA, 21 nt, Artificial Sequence
  siRNA passenger strand
gggagcugauggcguaggaaa

SEQ ID NO: 19 - RNA, 21 nt, Artificial Sequence
  siRNA guide strand (6)...(8) 2'-O-methyl modified
uccuacgccaucagcucccac

SEQ ID NO: 20 - RNA, 21 nt, Artificial Sequence
  siRNA passenger strand
gggagcugauggcguacgaaa

SEQ ID NO: 21 - RNA, 21 nt, Artificial Sequence
  siRNA guide strand
ucguacgccaucagcucccac

SEQ ID NO: 22 - RNA, 21 nt, Artificial Sequence
  siRNA passenger strand
gggagcugauggcguuggaaa

SEQ ID NO: 23 - RNA, 21 nt, Artificial Sequence
  siRNA guide strand
uccaacgccaucagcucccac

SEQ ID NO: 24 - RNA, 21 nt, Artificial Sequence
  siRNA passenger strand
gggagcugauggcgaaggaaa

SEQ ID NO: 25 - RNA, 21 nt, Artificial Sequence
  siRNA guide strand
uccuucgccaucagcucccac

SEQ ID NO: 26 - RNA, 21 nt, Artificial Sequence
  siRNA passenger strand
gggagcugauggccuaggaaa

SEQ ID NO: 27 - RNA, 21 nt, Artificial Sequence
  siRNA guide strand
uccuaggccaucagcucccac

SEQ ID NO: 28 - RNA, 21 nt, Artificial Sequence
  siRNA passenger strand
gggagcugaugggguaggaaa

SEQ ID NO: 29 - RNA, 21 nt, Artificial Sequence
  siRNA guide strand
uccuaccccaucagcucccac

SEQ ID NO: 30 - RNA, 21 nt, Artificial Sequence
  siRNA passenger strand
gggagcugauggcguacgaaa

SEQ ID NO: 31 - RNA, 21 nt, Artificial Sequence
  siRNA guide strand (6)...(8) 2'-O-methyl modified
ucguacgccaucagcucccac

SEQ ID NO: 32 - RNA, 21 nt, Artificial Sequence
  siRNA passenger strand
gggagcugauggcguuggaaa

SEQ ID NO: 33 - RNA, 21 nt, Artificial Sequence
  siRNA guide strand (6)...(8) 2'-O-methly modified
uccaacgccaucagcucccac

SEQ ID NO: 34 - RNA, 21 nt, Artificial Sequence
  siRNA
gggagcugauggcgaaggaaa

SEQ ID NO: 35 - RNA, 21 nt, Artificial Sequence
  siRNA guide strand (6)...(8) 2'-O-methyl modified
uccuucgccaucagcucccac

SEQ ID NO: 36 - RNA, 21 nt, Artificial Sequence
  siRNA passenger strand
gggagcugauggccuaggaaa

SEQ ID NO: 37 - RNA, 21 nt, Artificial Sequence
  siRNA guide strand (6)...(8) 2'-O-methyl modified
uccuaggccaucagcucccac

SEQ ID NO: 38 - RNA, 21 nt, Artificial Sequence
  siRNA passenger strand
gggagcugaugggguaggaaa

SEQ ID NO: 39 - RNA, 21 nt, Artificial Sequence
  siRNA guide strand (6)...(8) 2'-O-methyl modified
uccuaccccaucagcucccac

SEQ ID NO: 40 - RNA, 25 nt, Artificial Sequence
  reporter sense strand
cucaaccugcaccacgccuaggacg

SEQ ID NO: 41 - RNA, 21 nt, Artificial Sequence
  reporter antisense strand
uccuaggccaucagcucccac

SEQ ID NO: 42 - RNA, 21 nt, Artificial Sequence
  siRNA passenger strand
gggagcugauggccuaggaaa

SEQ ID NO: 43 - RNA, 21 nt, Artificial Sequence
  siRNA guide strand (6) and (8) 2'-O-methyl modified
uccuaggccaucagcucccac

SEQ ID NO: 44 - RNA, 21 nt, Artificial Sequence
  siRNA passenger strand
gggagcugauggcgaaggaaa

SEQ ID NO: 45 - RNA, 21 nt, Artificial Sequence
  siRNA guide strand (6) and (8) 2'-O-methyl modified
uccuucgccaucagcucccac

SEQ ID NO: 46 - RNA, 21 nt, Artificial Sequence
  siRNA passenger strand
gggagcuguuggcgaaggaaa

SEQ ID NO: 47 - RNA, 21 nt, Artificial Sequence
  siRNA guide strand (6) and (8) 2'-O-methyl modified
uccuucgccaacagcucccac

SEQ ID NO: 48 - RNA, 21 nt, Artificial Sequence
  siRNA passenger strand
gggagcuguuggccuaggaaa

SEQ ID NO: 49 - RNA, 21 nt, Artificial Sequence
  siRNA guide strand (6) and (8) 2'-O-methyl modified
uccuaggccaacagcucccac

SEQ ID NO: 50 - RNA, 21 nt, Artificial Sequence
  siRNA passenger strand
gggagcugcuggcgaaggaaa

SEQ ID NO: 51 - RNA, 21 nt, Artificial Sequence
  siRNA guide strand (6) and (8) 2'-O-methyl modified
uccuucgccagcagcucccac

SEQ ID NO: 52 - RNA, 21 nt, Artificial Sequence
  siRNA passenger strand
gggagcugcuggccuaggaaa

SEQ ID NO: 53 - RNA, 21 nt, Artificial Sequence
  siRNA guide strand (6) and (8) 2'-O-methyl modified
uccuaggccagcagcucccac

SEQ ID NO: 54 - RNA, 21 nt, Artificial Sequence
  siRNA passenger strand
cggagcagauggugauggaaa

SEQ ID NO: 55 - RNA, 21 nt, Artificial Sequence
  siRNA guide strand (6) and (8) 2'-O-methyl modified
uccaucaccaucugcuccgac

SEQ ID NO: 56 - RNA, 21 nt, Artificial Sequence
  siRNA passenger strand
ggcuggacgagaaguguaaag

SEQ ID NO: 57 - RNA, 21 nt, Artificial Sequence
  siRNA guide strand (6) and (8) 2'-O-methyl modified
uuacacuucucguccagccgu

SEQ ID NO: 58 - RNA, 21 nt, Artificial Sequence
  siRNA passenger strand
gcacaguaauucaucgcuaga

SEQ ID NO: 59 - RNA, 21 nt, Artificial Sequence
  siRNA guide strand (6) and (8) 2'-O-methyl modified
uagcgaugaauuacugugcgg

SEQ ID NO: 60 - RNA, 21 nt, Artificial Sequence
  siRNA passenger strand
gaagucugugcccaugugacc

SEQ ID NO: 61 - RNA, 21 nt, Artificial Sequence
  siRNA guide strand (6) and (8) 2'-O-methyl modified
ucacaugggcacagacuucca

SEQ ID NO: 62 - RNA, 21 nt, Artificial Sequence
  siRNA passenger strand
gccucauccacugagugcacu

SEQ ID NO: 63 - RNA, 21 nt, Artificial Sequence
  siRNA guide strand (6) and (8) 2'-O-methyl modified
ugcacucaguggaugaggcag

SEQ ID NO: 64 - RNA, 21 nt, Artificial Sequence
  siRNA passenger strand
ggcagcagcgggagcuauaag

SEQ ID NO: 65 - RNA, 21 nt, Artificial Sequence
  siRNA guide strand (6) and (8) 2'-O-methyl modified
uauagcucccgcugcugccgc

SEQ ID NO: 66 - RNA, 21 nt, Artificial Sequence
  siRNA passenger strand
gccacugguguggccagaacc

SEQ ID NO: 67 - RNA, 21 nt, Artificial Sequence
  siRNA guide strand (6) and (8) 2'-O-methyl modified
uucuggccacaccaguggcug

SEQ ID NO: 68 - RNA, 21 nt, Artificial Sequence
  siRNA passenger strand
gugccacugccacugcucauu

SEQ ID NO: 69 - RNA, 21 nt, Artificial Sequence
  siRNA guide strand (6) and (8) 2'-O-methyl modified
ugagcaguggcaguggcacca

SEQ ID NO: 70 - RNA, 21 nt, Artificial Sequence
  siRNA passenger strand
gcugcugaugggcucaccacu

SEQ ID NO: 71 - RNA, 21 nt, Artificial Sequence
  siRNA guide strand (6) and (8) 2'-O-methyl modified
uggugagcccaucagcagcag

SEQ ID NO: 72 - RNA, 21 nt, Artificial Sequence
  siRNA passenger strand
gccugguguucaugguggaag

SEQ ID NO: 73 - RNA, 21 nt, Artificial Sequence
  siRNA guide strand (6) and (8) 2'-O-methyl modified
gccaccaugaacaccaggccg

SEQ ID NO: 74 - RNA, 21 nt, Artificial Sequence
  siRNA passenger strand
gggcuuccucaacauacaagu

SEQ ID NO: 75 - RNA, 21 nt, Artificial Sequence
  siRNA guide strand (6) and (8) 2'-O-methyl modified
uuguauguugaggaagcccgg

SEQ ID NO: 76 - RNA, 21 nt, Artificial Sequence
  siRNA passenger strand
gcuuccacaagcgcuuccaau

SEQ ID NO: 77 - RNA, 21 nt, Artificial Sequence
  siRNA guide strand (6) and (8) 2'-O-methyl modified
uggaagcgcuuguggaagcug

SEQ ID NO: 78 - RNA, 21 nt, Artificial Sequence
  siRNA passenger strand
ggagcagccggccgagcuacg

SEQ ID NO: 79 - RNA, 21 nt, Artificial Sequence
  siRNA guide strand (6) and (8) 2'-O-methyl modified
uagcucggccggcugcuccuc

SEQ ID NO: 80 - RNA, 21 nt, Artificial Sequence
  siRNA passenger strand
gcacgugugucccagagaaca

SEQ ID NO: 81 - RNA, 21 nt, Artificial Sequence
  siRNA guide strand (6) and (8) 2'-O-methyl modified
uucucugggacacacgugcgg

SEQ ID NO: 82 - RNA, 21 nt, Artificial Sequence
  siRNA passenger strand
gcagcaacccccucagccagu

SEQ ID NO: 83 - RNA, 21 nt, Artificial Sequence
  siRNA guide strand (6) and (8) 2'-O-methyl modified
uggcugaggggguugcugcag

SEQ ID NO: 84 - RNA, 21 nt, Artificial Sequence
  siRNA passenger strand
gcacguccugggacgcggaag

SEQ ID NO: 85 - RNA, 21 nt, Artificial Sequence
  siRNA guide strand (6) and (8) 2'-O-methyl modified
uccgcgucccaggacgugcuu

SEQ ID NO: 86 - RNA, 21 nt, Artificial Sequence
  siRNA passenger strand
gccagggggaaugacuccacc

SEQ ID NO: 87 - RNA, 21 nt, Artificial Sequence
  siRNA guide strand (6) and (8) 2'-O-methyl modified
uggagucauucccccuggcuc

SEQ ID NO: 88 - RNA, 21 nt, Artificial Sequence
  siRNA passenger strand
ggcagcggcggcuccgggagg

SEQ ID NO: 89 - RNA, 21 nt, Artificial Sequence
  siRNA guide strand (6) and (8) 2'-O-methyl modified
ucccggagccgccgcugccgc

SEQ ID NO: 90 - RNA, 21 nt, Artificial Sequence
  siRNA passenger strand
gcgcagccacuuccaguaacc

SEQ ID NO: 91 - RNA, 21 nt, Artificial Sequence
  siRNA guide strand (6) and (8) 2'-O-methyl modified
uuacuggaaguggcugcgcac

SEQ ID NO: 92 - RNA, 21 nt, Artificial Sequence
  siRNA passenger strand
ggguggccucggcguaagacc

SEQ ID NO: 93 - RNA, 21 nt, Artificial Sequence
  siRNA guide strand (6) and (8) 2'-O-methyl modified
ucuuacgccgaggccacccgg

SEQ ID NO: 94 - RNA, 21 nt, Artificial Sequence
  siRNA passenger strand
gaguucucugagcuuugaaga

SEQ ID NO: 95 - RNA, 21 nt, Artificial Sequence
  siRNA guide strand (6) and (8) 2'-O-methyl modified
uucaaagcucagagaacucug

SEQ ID NO: 96 - RNA, 21 nt, Artificial Sequence
  siRNA passenger strand
gagcacacagucuacaguaaa

SEQ ID NO: 97 - RNA, 21 nt, Artificial Sequence
  siRNA guide strand (6) and (8) 2'-O-methyl modified
uacuguagacugugugcucuu

SEQ ID NO: 98 - RNA, 21 nt, Artificial Sequence
  siRNA passenger strand
gcagcccaggaccgggacacc

SEQ ID NO: 99 - RNA, 21 nt, Artificial Sequence
  siRNA guide strand (6) and (8) 2'-O-methyl modified
ugucccgguccugggcugcgg

SEQ ID NO: 100 - RNA, 21 nt, Artificial Sequence
  siRNA passenger strand
ggacccggacgccguggacca

SEQ ID NO: 101 - RNA, 21 nt, Artificial Sequence
  siRNA guide strand (6) and (8) 2'-O-methyl modified
uccagcugccacaggccccgg

SEQ ID NO: 102 - RNA, 21 nt, Artificial Sequence
  siRNA passenger strand
ggaauguggugcucguguauc

SEQ ID NO: 103 - RNA, 21 nt, Artificial Sequence
  siRNA guide strand (6) and (8) 2'-O-methyl modified
uacacgagcaccacauuccug

SEQ ID NO: 104 - RNA, 21 nt, Artificial Sequence
  siRNA passenger strand
gcaacaagguugcguccuaca

SEQ ID NO: 105 - RNA, 21 nt, Artificial Sequence
  siRNA guide strand (6) and (8) 2'-O-methyl modified
uaggacgcaaccuuguugcug

SEQ ID NO: 106 - RNA, 21 nt, Artificial Sequence
  siRNA passenger strand
gcuccagcuacuggagcaacu

SEQ ID NO: 107 - RNA, 21 nt, Artificial Sequence
  siRNA guide strand (6) and (8) 2'-O-methyl modified
uugcuccaguagcuggagcca